European Patent Specification EP 2 958 926 B1, published March 8, 2023. Title: EPIDITHIODIOXOPIPERAZINE COMPOUND OR ITS DERIVATIVES, AND THE USE THEREOF. Applicant: Ewha University - Industry Collaboration Foundation. The sequence listing filed with the application follows.

SEQUENCE LISTING (8 sequences)

SEQ ID NO: 1 - RNA, 21 nt, Artificial Sequence
  human PrxII siRNA-1
cgcuugucugaggauuacguu

SEQ ID NO: 2 - RNA, 21 nt, Artificial Sequence
  human PrxII siRNA-2
aggaauauuucuccaaacauu

SEQ ID NO: 3 - RNA, 21 nt, Artificial Sequence
  human PrxI siRNA
actcaactgccaagtgattuu

SEQ ID NO: 4 - RNA, 21 nt, Artificial Sequence
  mouse PrxII siRNA-1
aggaauauuucuccaaacauu

SEQ ID NO: 5 - RNA, 21 nt, Artificial Sequence
  siRNA for Rat PrxII
gcaacgcgcacaucggaaauu

SEQ ID NO: 6 - RNA, 21 nt, Artificial Sequence
  siRNA for Rat PrxII
gaucacagucaacgaccuauu

SEQ ID NO: 7 - RNA, 21 nt, Artificial Sequence
  siRNA for Rat PrxII
agaauuacggcguguugaauu

SEQ ID NO: 8 - RNA, 21 nt, Artificial Sequence
  siRNA for Rat PrxII
acgcugaggacuuccgaaauu